European Patent Specification EP 4 072 520 B1, published September 24, 2025. Title: COMPOSITION. Applicant: ViiV Healthcare Company. The sequence listing filed with the application follows.

SEQUENCE LISTING (2 sequences)

SEQ ID NO: 1 - protein, 121 aa, Human
RAHLVQSGTAMKKPGASVRVSCQTSGYTFTAHILFWFRQAPGRGLEWVGWIKPQYGAVNFGGGFRDRVTLTRDVYREIAYMDIRGLKPDDTAVYYCARDRSYGDSSWALDAWGQGTTVWSA

SEQ ID NO: 2 - protein, 103 aa, Human [sequence omitted]